European Patent Application EP 4 559 933 A1, published May 28, 2025. Title: 促进多特异性抗体的重链和轻链同源配对的突变体. Applicant: 信达生物制药（苏州）有限公司. The sequence listing filed with the application follows.

SEQUENCE LISTING (152 sequences)

SEQ ID NO: 1 - protein, 103 aa, artificial sequence
ASTKGPSVCPLAPSSKSTSGGTAALGCLVKDYFPEPVTVSWNSGALTSGVHTFPAVLQSSGLYSLSSVVTVPSSSLGTQTYICNVNHKPSNTKVDKKVEPKSC

SEQ ID NO: 2 - protein, 107 aa, artificial sequence
RTVAAPSVFIFPPSDECLKSGTASVVCLLNNFYPREAKVQWKVDNALQSGNSQESVTEQDSKDSTYSLSSTLTLSKADYEKHKVYACEVTHQGLSSPVTKSFNRGEC

SEQ ID NO: 3 - protein, 120 aa, artificial sequence
EVQLVESGGGLVQPGGSLRLSCAASGFNIKDTYIHWVRKAPGKGLEWVARIYPTNGYTRYADSVKGRFTISADTSKNTAYLQMNSLRAEDTAVYYCSRWGGDGFYAMDYWGQGTLVTVSS

SEQ ID NO: 4 - protein, 107 aa, artificial sequence
DIQMTQSPSSLSASVGDRVTITCRASQDVNTAVAWYQDKPGKAPKLLIYSASFLYSGVPSRFSGSRSGTDFTLTISSLQPEDFATYYCQQHYTTPPTFGQGTKVEIK

SEQ ID NO: 5 - protein, 119 aa, artificial sequence
EVRLLESGGGLVQPGGSLRLSCAASGFTFSNYAMGWVRDAPGKGLEWVSAISGSGGSTYYADSVKGRFTTSRDDSKNALYLQMNSLRAEDTAVYYCARGGPGWYAADVWGQGTTVTVSS

SEQ ID NO: 6 - protein, 107 aa, artificial sequence
DIQMTQSPSSLSASVGDRVTITCRASQSISSYLNWYQKKPGKAPKLLIYAASSLQSGVPSRFSGSGSGTDFTLTISSLQPEDFATYYCQQADLPAFAFGGGTKVEIK

SEQ ID NO: 7 - protein, 120 aa, artificial sequence
EVQLVESGGGLVQPGGSLRLSCAASGFNIKDTYIHWVRQAPGKGKEWVARIYPTNGYTRYADSVKGRFTISADTSKNTAYLQMNSLRAEDTAVYYCSRWGGDGFYAMDYWGQGTLVTVSS

SEQ ID NO: 8 - protein, 107 aa, artificial sequence
DIQMTQSPSSLSASVGDRVTITCRASQDVNTAVAWYQQKPGKAPKLLIYSASFLYSGVPSRFSGSRSGTDFTLTISSLQPEDFATYDCQQHYTTPPTFGQGTKVEIK

SEQ ID NO: 9 - protein, 119 aa, artificial sequence
EVRLLESGGGLVQPGGSLRLSCAASGFTFSNYAMGWVRQAPGKGDEWVSAISGSGGSTYYADSVKGRFTTSRDDSKNALYLQMNSLRAEDTAVYYCARGGPGWYAADVWGQGTTVTVSS

SEQ ID NO: 10 - protein, 107 aa, artificial sequence
DIQMTQSPSSLSASVGDRVTITCRASQSISSYLNWYQQKPGKAPKLLIYAASSLQSGVPSRFSGSGSGTDFTLTISSLQPEDFATYKCQQADLPAFAFGGGTKVEIK

SEQ ID NO: 11 - protein, 107 aa, artificial sequence
DIQMTQSPSSLSASVGDRVTITCRASQDVNTAVAWYQQKPGKADKLLIYSASFLYSGVPSRFSGSRSGTDFTLTISSLQPEDFATYYCQQHYTTPPTFGQGTKVEIK

SEQ ID NO: 12 - protein, 107 aa, artificial sequence
DIQMTQSPSSLSASVGDRVTITCRASQSISSYLNWYQQKPGKAKKLLIYAASSLQSGVPSRFSGSGSGTDFTLTISSLQPEDFATYYCQQADLPAFAFGGGTKVEIK

SEQ ID NO: 13 - protein, 120 aa, artificial sequence
EVQLVESGGGLVQPGGSLRLSCAASGFNIKDTYIHWVRQAPGKGLEWVARIYPTNGYTRYADSVKGRFTISADTSKNTAYLQMNSLRAEDTAVYKCSRWGGDGFYAMDYWGQGTLVTVSS

SEQ ID NO: 14 - protein, 107 aa, artificial sequence
DIQMTQSPSSLSASVGDRVTITCRASQDVNTAVAWYQQKPGKDPKLLIYSASFLYSGVPSRFSGSRSGTDFTLTISSLQPEDFATYYCQQHYTTPPTFGQGTKVEIK

SEQ ID NO: 15 - protein, 119 aa, artificial sequence
EVRLLESGGGLVQPGGSLRLSCAASGFTFSNYAMGWVRQAPGKGLEWVSAISGSGGSTYYADSVKGRFTTSRDDSKNALYLQMNSLRAEDTAVYDCARGGPGWYAADVWGQGTTVTVSS

SEQ ID NO: 16 - protein, 107 aa, artificial sequence
DIQMTQSPSSLSASVGDRVTITCRASQSISSYLNWYQQKPGKKPKLLIYAASSLQSGVPSRFSGSGSGTDFTLTISSLQPEDFATYYCQQADLPAFAFGGGTKVEIK

SEQ ID NO: 17 - protein, 113 aa, artificial sequence [sequence omitted]

SEQ ID NO: 18 - protein, 119 aa, artificial sequence [sequence omitted]

SEQ ID NO: 19 - protein, 111 aa, artificial sequence
DIVMTQSPDSLAVSLGERATINCRASESVDSYGITFMNWYQDKPGQPPKLLIYAASNQGSGVPDRFSGSGSGTDFTLTISSLQAEDVAVYYCQQSKEVPWTFGQGTKLEIK

SEQ ID NO: 20 - protein, 227 aa, artificial sequence [sequence omitted]

SEQ ID NO: 21 - protein, 450 aa, artificial sequence
EVQLVESGGGLVQPGGSLRLSCAASGFNIKDTYIHWVRKAPGKGLEWVARIYPTNGYTRYADSVKGRFTISADTSKNTAYLQMNSLRAEDTAVYYCSRWGGDGFYAMDYWGQGTLVTVSSASTKGPSVCPLAPSSKSTSGGTAALGCLVKDYFPEPVTVSWNSGALTSGVHTFPAVLQSSGLYSLSSVVTVPSSSLGTQTYICNVNHKPSNTKVDKKVEPKSSDKTHTCPPCPAPEAAGGPSVFLFPPKPKDTLMISRTPEVTCVVVDVSHEDPEVKFNWYVDGVEVHNAKTKPREEQYNSTYRVVSVLTVLHQDWLNGKEYKCKVSNKALPAPIEKTISKAKGQPREPQVYTLPPCRDELTKNQVSLWCLVKGFYPSDIAVEWESNGQPENNYKTTPPVLDSDGSFFLYSKLTVDKSRWQQGNVFSCSVMHEALHNHYTQKSLSLSPGK

SEQ ID NO: 22 - protein, 214 aa, artificial sequence
DIQMTQSPSSLSASVGDRVTITCRASQDVNTAVAWYQDKPGKAPKLLIYSASFLYSGVPSRFSGSRSGTDFTLTISSLQPEDFATYYCQQHYTTPPTFGQGTKVEIKRTVAAPSVFIFPPSDECLKSGTASVVCLLNNFYPREAKVQWKVDNALQSGNSQESVTEQDSKDSTYSLSSTLTLSKADYEKHKVYACEVTHQGLSSPVTKSFNRGES

SEQ ID NO: 23 - protein, 449 aa, artificial sequence
EVRLLESGGGLVQPGGSLRLSCAASGFTFSNYAMGWVRDAPGKGLEWVSAISGSGGSTYYADSVKGRFTTSRDDSKNALYLQMNSLRAEDTAVYYCARGGPGWYAADVWGQGTTVTVSSASTKGPSVFPLAPSSKSTSGGTAALGCLVKDYFPEPVTVSWNSGALTSGVHTFPAVLQSSGLYSLSSVVTVPSSSLGTQTYICNVNHKPSNTKVDKKVEPKSCDKTHTCPPCPAPEAAGGPSVFLFPPKPKDTLMISRTPEVTCVVVDVSHEDPEVKFNWYVDGVEVHNAKTKPREEQYNSTYRVVSVLTVLHQDWLNGKEYKCKVSNKALPAPIEKTISKAKGQPREPQVCTLPPSRDELTKNQVSLSCAVKGFYPSDIAVEWESNGQPENNYKTTPPVLDSDGSFFLVSKLTVDKSRWQQGNVFSCSVMHEALHNHYTQKSLSLSPGK

SEQ ID NO: 24 - protein, 214 aa, artificial sequence
DIQMTQSPSSLSASVGDRVTITCRASQSISSYLNWYQKKPGKAPKLLIYAASSLQSGVPSRFSGSGSGTDFTLTISSLQPEDFATYYCQQADLPAFAFGGGTKVEIKRTVAAPSVFIFPPSDEQLKSGTASVVCLLNNFYPREAKVQWKVDNALQSGNSQESVTEQDSKDSTYSLSSTLTLSKADYEKHKVYACEVTHQGLSSPVTKSFNRGEC

SEQ ID NO: 25 - protein, 450 aa, artificial sequence
EVQLVESGGGLVQPGGSLRLSCAASGFNIKDTYIHWVRQAPGKGKEWVARIYPTNGYTRYADSVKGRFTISADTSKNTAYLQMNSLRAEDTAVYYCSRWGGDGFYAMDYWGQGTLVTVSSASTKGPSVCPLAPSSKSTSGGTAALGCLVKDYFPEPVTVSWNSGALTSGVHTFPAVLQSSGLYSLSSVVTVPSSSLGTQTYICNVNHKPSNTKVDKKVEPKSSDKTHTCPPCPAPEAAGGPSVFLFPPKPKDTLMISRTPEVTCVVVDVSHEDPEVKFNWYVDGVEVHNAKTKPREEQYNSTYRVVSVLTVLHQDWLNGKEYKCKVSNKALPAPIEKTISKAKGQPREPQVYTLPPCRDELTKNQVSLWCLVKGFYPSDIAVEWESNGQPENNYKTTPPVLDSDGSFFLYSKLTVDKSRWQQGNVFSCSVMHEALHNHYTQKSLSLSPGK

SEQ ID NO: 26 - protein, 214 aa, artificial sequence
DIQMTQSPSSLSASVGDRVTITCRASQDVNTAVAWYQQKPGKAPKLLIYSASFLYSGVPSRFSGSRSGTDFTLTISSLQPEDFATYDCQQHYTTPPTFGQGTKVEIKRTVAAPSVFIFPPSDECLKSGTASVVCLLNNFYPREAKVQWKVDNALQSGNSQESVTEQDSKDSTYSLSSTLTLSKADYEKHKVYACEVTHQGLSSPVTKSFNRGES

SEQ ID NO: 27 - protein, 449 aa, artificial sequence
EVRLLESGGGLVQPGGSLRLSCAASGFTFSNYAMGWVRQAPGKGDEWVSAISGSGGSTYYADSVKGRFTTSRDDSKNALYLQMNSLRAEDTAVYYCARGGPGWYAADVWGQGTTVTVSSASTKGPSVFPLAPSSKSTSGGTAALGCLVKDYFPEPVTVSWNSGALTSGVHTFPAVLQSSGLYSLSSVVTVPSSSLGTQTYICNVNHKPSNTKVDKKVEPKSCDKTHTCPPCPAPEAAGGPSVFLFPPKPKDTLMISRTPEVTCVVVDVSHEDPEVKFNWYVDGVEVHNAKTKPREEQYNSTYRVVSVLTVLHQDWLNGKEYKCKVSNKALPAPIEKTISKAKGQPREPQVCTLPPSRDELTKNQVSLSCAVKGFYPSDIAVEWESNGQPENNYKTTPPVLDSDGSFFLVSKLTVDKSRWQQGNVFSCSVMHEALHNHYTQKSLSLSPGK

SEQ ID NO: 28 - protein, 214 aa, artificial sequence
DIQMTQSPSSLSASVGDRVTITCRASQSISSYLNWYQQKPGKAPKLLIYAASSLQSGVPSRFSGSGSGTDFTLTISSLQPEDFATYKCQQADLPAFAFGGGTKVEIKRTVAAPSVFIFPPSDEQLKSGTASVVCLLNNFYPREAKVQWKVDNALQSGNSQESVTEQDSKDSTYSLSSTLTLSKADYEKHKVYACEVTHQGLSSPVTKSFNRGEC

SEQ ID NO: 29 - protein, 214 aa, artificial sequence
DIQMTQSPSSLSASVGDRVTITCRASQDVNTAVAWYQQKPGKADKLLIYSASFLYSGVPSRFSGSRSGTDFTLTISSLQPEDFATYYCQQHYTTPPTFGQGTKVEIKRTVAAPSVFIFPPSDECLKSGTASVVCLLNNFYPREAKVQWKVDNALQSGNSQESVTEQDSKDSTYSLSSTLTLSKADYEKHKVYACEVTHQGLSSPVTKSFNRGES

SEQ ID NO: 30 - protein, 214 aa, artificial sequence
DIQMTQSPSSLSASVGDRVTITCRASQSISSYLNWYQQKPGKAKKLLIYAASSLQSGVPSRFSGSGSGTDFTLTISSLQPEDFATYYCQQADLPAFAFGGGTKVEIKRTVAAPSVFIFPPSDEQLKSGTASVVCLLNNFYPREAKVQWKVDNALQSGNSQESVTEQDSKDSTYSLSSTLTLSKADYEKHKVYACEVTHQGLSSPVTKSFNRGEC

SEQ ID NO: 31 - protein, 450 aa, artificial sequence
EVQLVESGGGLVQPGGSLRLSCAASGFNIKDTYIHWVRQAPGKGLEWVARIYPTNGYTRYADSVKGRFTISADTSKNTAYLQMNSLRAEDTAVYKCSRWGGDGFYAMDYWGQGTLVTVSSASTKGPSVCPLAPSSKSTSGGTAALGCLVKDYFPEPVTVSWNSGALTSGVHTFPAVLQSSGLYSLSSVVTVPSSSLGTQTYICNVNHKPSNTKVDKKVEPKSSDKTHTCPPCPAPEAAGGPSVFLFPPKPKDTLMISRTPEVTCVVVDVSHEDPEVKFNWYVDGVEVHNAKTKPREEQYNSTYRVVSVLTVLHQDWLNGKEYKCKVSNKALPAPIEKTISKAKGQPREPQVYTLPPCRDELTKNQVSLWCLVKGFYPSDIAVEWESNGQPENNYKTTPPVLDSDGSFFLYSKLTVDKSRWQQGNVFSCSVMHEALHNHYTQKSLSLSPGK

SEQ ID NO: 32 - protein, 214 aa, artificial sequence
DIQMTQSPSSLSASVGDRVTITCRASQDVNTAVAWYQQKPGKDPKLLIYSASFLYSGVPSRFSGSRSGTDFTLTISSLQPEDFATYYCQQHYTTPPTFGQGTKVEIKRTVAAPSVFIFPPSDECLKSGTASVVCLLNNFYPREAKVQWKVDNALQSGNSQESVTEQDSKDSTYSLSSTLTLSKADYEKHKVYACEVTHQGLSSPVTKSFNRGES

SEQ ID NO: 33 - protein, 449 aa, artificial sequence
EVRLLESGGGLVQPGGSLRLSCAASGFTFSNYAMGWVRQAPGKGLEWVSAISGSGGSTYYADSVKGRFTTSRDDSKNALYLQMNSLRAEDTAVYDCARGGPGWYAADVWGQGTTVTVSSASTKGPSVFPLAPSSKSTSGGTAALGCLVKDYFPEPVTVSWNSGALTSGVHTFPAVLQSSGLYSLSSVVTVPSSSLGTQTYICNVNHKPSNTKVDKKVEPKSCDKTHTCPPCPAPEAAGGPSVFLFPPKPKDTLMISRTPEVTCVVVDVSHEDPEVKFNWYVDGVEVHNAKTKPREEQYNSTYRVVSVLTVLHQDWLNGKEYKCKVSNKALPAPIEKTISKAKGQPREPQVCTLPPSRDELTKNQVSLSCAVKGFYPSDIAVEWESNGQPENNYKTTPPVLDSDGSFFLVSKLTVDKSRWQQGNVFSCSVMHEALHNHYTQKSLSLSPGK

SEQ ID NO: 34 - protein, 214 aa, artificial sequence
DIQMTQSPSSLSASVGDRVTITCRASQSISSYLNWYQQKPGKKPKLLIYAASSLQSGVPSRFSGSGSGTDFTLTISSLQPEDFATYYCQQADLPAFAFGGGTKVEIKRTVAAPSVFIFPPSDEQLKSGTASVVCLLNNFYPREAKVQWKVDNALQSGNSQESVTEQDSKDSTYSLSSTLTLSKADYEKHKVYACEVTHQGLSSPVTKSFNRGEC

SEQ ID NO: 35 - protein, 107 aa, artificial sequence
RTVAAPSVFIFPPSDEQLKSGTASVVCLLNNFYPREAKVQWKVDNALQSGNSCESVTEQDSKDSTYSLSSTLTLSKADYEKHKVYACEVTHQGLSSPVTKSFNRGES

SEQ ID NO: 36 - protein, 107 aa, artificial sequence
RTVAAPSVFICPPSDEQLKSGTASVVCLLNNFYPREAKVQWKVDNALQSGNSQESVTEQDSKDSTYSLSSTLTLSKADYEKHKVYACEVTHQGLSSPVTKSFNRGEC

SEQ ID NO: 37 - protein, 107 aa, artificial sequence
RTVAAPSVFICPPSDEQLKSGTASVVCLLNNFYPREAKVQWKVDNALQSGNSQESVTEQDSKDSTYSLSSTLTLSKADYEKHKVYACEVTHQGLSSPVTKSFNRGES

SEQ ID NO: 38 - protein, 107 aa, artificial sequence
RTVAAPSVCIFPPSDEQLKSGTASVVCLLNNFYPREAKVQWKVDNALQSGNSQESVTEQDSKDSTYSLSSTLTLSKADYEKHKVYACEVTHQGLSSPVTKSFNRGEC

SEQ ID NO: 39 - protein, 450 aa, artificial sequence
EVQLVESGGGLVQPGGSLRLSCAASGFNIKDTYIHWVRQAPGKGLEWVARIYPTNGYTRYADSVKGRFTISADTSKNTAYLQMNSLRAEDTAVYYCSRWGGDGFYAMDYWGQGTLVTVSSASTKGPSVFPLAPSSKSTSGGTAALGCLVKDYFPEPVTVSWNSGALTSGVHTFPAVLQSSGLYSLSSVVTVPSSSLGTQTYICNVNHKPSNTKVDKKVEPKSCDKTHTCPPCPAPEAAGGPSVFLFPPKPKDTLMISRTPEVTCVVVDVSHEDPEVKFNWYVDGVEVHNAKTKPREEQYNSTYRVVSVLTVLHQDWLNGKEYKCKVSNKALPAPIEKTISKAKGQPREPQVYTLPPCRDELTKNQVSLWCLVKGFYPSDIAVEWESNGQPENNYKTTPPVLDSDGSFFLYSKLTVDKSRWQQGNVFSCSVMHEALHNHYTQKSLSLSPGK

SEQ ID NO: 40 - protein, 214 aa, artificial sequence
DIQMTQSPSSLSASVGDRVTITCRASQDVNTAVAWYQQKPGKAPKLLIYSASFLYSGVPSRFSGSRSGTDFTLTISSLQPEDFATYYCQQHYTTPPTFGQGTKVEIKRTVAAPSVFIFPPSDEQLKSGTASVVCLLNNFYPREAKVQWKVDNALQSGNSQESVTEQDSKDSTYSLSSTLTLSKADYEKHKVYACEVTHQGLSSPVTKSFNRGEC

SEQ ID NO: 41 - protein, 449 aa, artificial sequence
EVRLLESGGGLVQPGGSLRLSCAASGFTFSNYAMGWVRQAPGKGLEWVSAISGSGGSTYYADSVKGRFTTSRDDSKNALYLQMNSLRAEDTAVYYCARGGPGWYAADVWGQGTTVTVSSASTKGPSVFPLAPSSKSTSGGTAALGCLVKDYFPEPVTVSWNSGALTSGVHTFPAVLQSSGLYSLSSVVTVPSSSLGTQTYICNVNHKPSNTKVDKKVEPKSCDKTHTCPPCPAPEAAGGPSVFLFPPKPKDTLMISRTPEVTCVVVDVSHEDPEVKFNWYVDGVEVHNAKTKPREEQYNSTYRVVSVLTVLHQDWLNGKEYKCKVSNKALPAPIEKTISKAKGQPREPQVCTLPPSRDELTKNQVSLSCAVKGFYPSDIAVEWESNGQPENNYKTTPPVLDSDGSFFLVSKLTVDKSRWQQGNVFSCSVMHEALHNHYTQKSLSLSPGK

SEQ ID NO: 42 - protein, 214 aa, artificial sequence
DIQMTQSPSSLSASVGDRVTITCRASQSISSYLNWYQQKPGKAPKLLIYAASSLQSGVPSRFSGSGSGTDFTLTISSLQPEDFATYYCQQADLPAFAFGGGTKVEIKRTVAAPSVFIFPPSDEQLKSGTASVVCLLNNFYPREAKVQWKVDNALQSGNSQESVTEQDSKDSTYSLSSTLTLSKADYEKHKVYACEVTHQGLSSPVTKSFNRGEC

SEQ ID NO: 43 - protein, 450 aa, artificial sequence
EVQLVESGGGLVQPGGSLRLSCAASGFNIKDTYIHWVRQAPGKGLEWVARIYPTNGYTRYADSVKGRFTISADTSKNTAYLQMNSLRAEDTAVYYCSRWGGDGFYAMDYWGQGTLVTVSSASTKGPSVCPLAPSSKSTSGGTAALGCLVKDYFPEPVTVSWNSGALTSGVHTFPAVLQSSGLYSLSSVVTVPSSSLGTQTYICNVNHKPSNTKVDKKVEPKSCDKTHTCPPCPAPEAAGGPSVFLFPPKPKDTLMISRTPEVTCVVVDVSHEDPEVKFNWYVDGVEVHNAKTKPREEQYNSTYRVVSVLTVLHQDWLNGKEYKCKVSNKALPAPIEKTISKAKGQPREPQVYTLPPCRDELTKNQVSLWCLVKGFYPSDIAVEWESNGQPENNYKTTPPVLDSDGSFFLYSKLTVDKSRWQQGNVFSCSVMHEALHNHYTQKSLSLSPGK

SEQ ID NO: 44 - protein, 214 aa, artificial sequence
DIQMTQSPSSLSASVGDRVTITCRASQDVNTAVAWYQQKPGKAPKLLIYSASFLYSGVPSRFSGSRSGTDFTLTISSLQPEDFATYYCQQHYTTPPTFGQGTKVEIKRTVAAPSVFIFPPCDEQLKSGTASVVCLLNNFYPREAKVQWKVDNALQSGNSQESVTEQDSKDSTYSLSSTLTLSKADYEKHKVYACEVTHQGLSSPVTKSFNRGEC

SEQ ID NO: 45 - protein, 214 aa, artificial sequence
DIQMTQSPSSLSASVGDRVTITCRASQDVNTAVAWYQQKPGKAPKLLIYSASFLYSGVPSRFSGSRSGTDFTLTISSLQPEDFATYYCQQHYTTPPTFGQGTKVEIKRTVAAPSVFIFPPSDECLKSGTASVVCLLNNFYPREAKVQWKVDNALQSGNSQESVTEQDSKDSTYSLSSTLTLSKADYEKHKVYACEVTHQGLSSPVTKSFNRGEC

SEQ ID NO: 46 - protein, 450 aa, artificial sequence
QVQLVQSGAEVKKPGSSVKVSCKASGGTFSSYAISWVRQAPGQGLEWMGLIIPMFDTAGYAQKFQGRVAITVDESTSTAYMELSSLRSEDTAVYYCARAEHSSTGTFDYWGQGTLVTVSSASTKGPSVFPLAPSSKSTSGGTAALGCLVKDYFPEPVTVSWNSGALTSGVHTFPAVLQSSGLYSLSSVVTVPSSSLGTQTYICNVNHKPSNTKVDKKVEPKSCDKTHTCPPCPAPEAAGGPSVFLFPPKPKDTLMISRTPEVTCVVVDVSHEDPEVKFNWYVDGVEVHNAKTKPREEQYNSTYRVVSVLTVLHQDWLNGKEYKCKVSNKALPAPIEKTISKAKGQPREPQVCTLPPSRDELTKNQVSLSCAVKGFYPSDIAVEWESNGQPENNYKTTPPVLDSDGSFFLVSKLTVDKSRWQQGNVFSCSVMHEALHNHYTQKSLSLSPGK

SEQ ID NO: 47 - protein, 214 aa, artificial sequence
DIQMTQSPSSVSASVGDRVTITCRASQGISSWLAWYQQKPGKAPKLLISAASSLQSGVPSRFSGSGSGTDFTLTISSLQPEDFATYYCQQANHLPFTFGGGTKVEIKRTVAAPSVFIFPPSDEQLKSGTASVVCLLNNFYPREAKVQWKVDNALQSGNSQESVTEQDSKDSTYSLSSTLTLSKADYEKHKVYACEVTHQGLSSPVTKSFNRGEC

SEQ ID NO: 48 - protein, 450 aa, artificial sequence
EVQLVESGGGLVQPGGSLRLSCAASGFNIKDTYIHWVRQAPGKGLEWVARIYPTNGYTRYADSVKGRFTISADTSKNTAYLQMNSLRAEDTAVYYCSRWGGDGFYAMDYWGQGTLVTVSSASTKGPSVCPLAPSSKSTSGGTAALGCLVKDYFPEPVTVSWNSGALTSGVHTFPAVLQSSGLYSLSSVVTVPSSSLGTQTYICNVNHKPSNTKVDKKVEPKSSDKTHTCPPCPAPEAAGGPSVFLFPPKPKDTLMISRTPEVTCVVVDVSHEDPEVKFNWYVDGVEVHNAKTKPREEQYNSTYRVVSVLTVLHQDWLNGKEYKCKVSNKALPAPIEKTISKAKGQPREPQVYTLPPCRDELTKNQVSLWCLVKGFYPSDIAVEWESNGQPENNYKTTPPVLDSDGSFFLYSKLTVDKSRWQQGNVFSCSVMHEALHNHYTQKSLSLSPGK

SEQ ID NO: 49 - protein, 214 aa, artificial sequence
DIQMTQSPSSLSASVGDRVTITCRASQDVNTAVAWYQQKPGKAPKLLIYSASFLYSGVPSRFSGSRSGTDFTLTISSLQPEDFATYYCQQHYTTPPTFGQGTKVEIKRTVAAPSVFIFPPSDECLKSGTASVVCLLNNFYPREAKVQWKVDNALQSGNSQESVTEQDSKDSTYSLSSTLTLSKADYEKHKVYACEVTHQGLSSPVTKSFNRGES

SEQ ID NO: 50 - protein, 445 aa, artificial sequence
QVQLQESGPGLVKPSETLSLTCTVSGGSISSYYWSWIRQPPGKGLEWIGYIYYSGSTNYNPSLKSRVTISVDTSKNQFSLKLSSVTAADTAVYYCARGKTGSAAWGQGTLVTVSSASTKGPSVFPLAPSSKSTSGGTAALGCLVKDYFPEPVTVSWNSGALTSGVHTFPAVLQSSGLYSLSSVVTVPSSSLGTQTYICNVNHKPSNTKVDKKVEPKSCDKTHTCPPCPAPEAAGGPSVFLFPPKPKDTLMISRTPEVTCVVVDVSHEDPEVKFNWYVDGVEVHNAKTKPREEQYNSTYRVVSVLTVLHQDWLNGKEYKCKVSNKALPAPIEKTISKAKGQPREPQVCTLPPSRDELTKNQVSLSCAVKGFYPSDIAVEWESNGQPENNYKTTPPVLDSDGSFFLVSKLTVDKSRWQQGNVFSCSVMHEALHNHYTQKSLSLSPGK

SEQ ID NO: 51 - protein, 214 aa, artificial sequence
DIQMTQSPSSVSASVGDRVTITCRASQGISRWLAWYQQKPGKAPKLLIYAASSLQSGVPSRFSGSGSGTDFTLTISSLQPEDFATYYCQQTVSFPITFGGGTKVEIKRTVAAPSVFIFPPSDEQLKSGTASVVCLLNNFYPREAKVQWKVDNALQSGNSQESVTEQDSKDSTYSLSSTLTLSKADYEKHKVYACEVTHQGLSSPVTKSFNRGEC

SEQ ID NO: 52 - protein, 449 aa, artificial sequence
EVQLVESGGGLVQPGGSLRLSCAASGYTFTSYWLHWVRQAPGKGLEWVGMIDPSNSDTRFNPNFKDRFTISADTSKNTAYLQMNSLRAEDTAVYYCATYRSYVTPLDYWGQGTLVTVSSASTKGPSVFPLAPSSKSTSGGTAALGCLVKDYFPEPVTVSWNSGALTSGVHTFPAVLQSSGLYSLSSVVTVPSSSLGTQTYICNVNHKPSNTKVDKKVEPKSCDKTHTCPPCPAPEAAGGPSVFLFPPKPKDTLMISRTPEVTCVVVDVSHEDPEVKFNWYVDGVEVHNAKTKPREEQYNSTYRVVSVLTVLHQDWLNGKEYKCKVSNKALPAPIEKTISKAKGQPREPQVCTLPPSRDELTKNQVSLSCAVKGFYPSDIAVEWESNGQPENNYKTTPPVLDSDGSFFLVSKLTVDKSRWQQGNVFSCSVMHEALHNHYTQKSLSLSPGK

SEQ ID NO: 53 - protein, 220 aa, artificial sequence
DIQMTQSPSSLSASVGDRVTITCKSSQSLLYTSSQKNYLAWYQQKPGKAPKLLIYWASTRESGVPSRFSGSGSGTDFTLTISSLQPEDFATYYCQQYYAYPWTFGQGTKVEIKRTVAAPSVFIFPPSDEQLKSGTASVVCLLNNFYPREAKVQWKVDNALQSGNSQESVTEQDSKDSTYSLSSTLTLSKADYEKHKVYACEVTHQGLSSPVTKSFNRGEC

SEQ ID NO: 54 - protein, 107 aa, artificial sequence [sequence omitted]

SEQ ID NO: 55 - protein, 106 aa, artificial sequence
GQPKAAPSVTLFPPSSEELQANKATLVCLISDFYPGAVTVAWKADSSPVKAGVETTTPSKQSNNKYAASSYLSLTPEQWKSHRSYSCQVTHEGSTVEKTVAPTECS

SEQ ID NO: 56 - protein, 218 aa, artificial sequence
DIVMTQSPDSLAVSLGERATINCRASESVDSYGITFMNWYQQKPGQPPKLLIYAASNQGSGVPDRFSGSGSGTDFTLTISSLQAEDVAVYYCQQSKEVPWTFGQGTKLEIKRTVAAPSVFIFPPSDEQLKSGTASVVCLLNNFYPREAKVQWKVDNALQSGNSQESVTEQDSKDSTYSLSSTLTLSKADYEKHKVYACEVTHQGLSSPVTKSFNRGEC

SEQ ID NO: 57 - protein, 450 aa, artificial sequence
QVQLVQSGAEVKKPGASVKVSCKASGYTFIGYVMHWVRQAPGQGLEWMGYINPYNDVSQHQGKFKGRVTMTSDTSTSTVYMELSSLRSEDTAVYYCAREGRLGLRVLAYWGQGTLVTVSSASTKGPSVFPLAPSSKSTSGGTAALGCLVKDYFPEPVTVSWNSGALTSGVHTFPAVLQSSGLYSLSSVVTVPSSSLGTQTYICNVNHKPSNTKVDKKVEPKSCDKTHTCPPCPAPELLGGPSVFLFPPKPKDTLMISRTPEVTCVVVDVSHEDPEVKFNWYVDGVEVHNAKTKPREEQYNSTYRVVSVLTVLHQDWLNGKEYKCKVSNKALPAPIEKTISKAKGQPREPQVYTLPPSREEMTKNQVRLTCLVKGFYPSDIAVEWESNGQPENNYKTTPPVLKSDGSFFLYSKLTVDKSRWQQGNVFSCSVMHEALHNHYTQKSLSLSPGK

SEQ ID NO: 58 - protein, 688 aa, artificial sequence
QVQLVQSGAEVKKPGASVKVSCKASGYTFIGYVMHWVRQAPGQGLEWMGYINPYNDVSQHQGKFKGRVTMTSDTSTSTVYMELSSLRSEDTAVYYCAREGRLGLRVLAYWGQGTLVTVSSASTKGPSVFPLAPSSKSTSGGTAALGCLVKDYFPEPVTVSWNSGALTSGVHTFPAVLQSSGLYSLSSVVTVPSSSLGTQTYICNVNHKPSNTKVDKKVEPKSCGGGGSGGGGSEVQLVESGGGLVQPGGSLKLSCAASGFTFNTYAMNWVRQASGKGLEWVGRIRSKYNNYATYYADSVKDRFTISRDDSKSTLYLQMNSLKTEDTAVYYCARHGNFGQSYVSWFAYWGQGTTVTVSSASTKGPSVCPLAPSSKSTSGGTAALGCLVKDYFPEPVTVSWNSGALTSGVHTFPAVLQSSGLYSLSSVVTVPSSSLGTQTYICNVNHKPSNTKVDKKVEPKSSDKTHTCPPCPAPELLGGPSVFLFPPKPKDTLMISRTPEVTCVVVDVSHEDPEVKFNWYVDGVEVHNAKTKPREEQYNSTYRVVSVLTVLHQDWLNGKEYKCKVSNKALPAPIEKTISKAKGQPREPQVTTLPPSREEMTKNQVSLTCLVSGFYPSDIAVEWESNGQPENNYKTTPPVLDSDGSFFLYSDLTVDKSRWQQGNVFSCSVMHEALHNHYTQKSLSLSPGK

SEQ ID NO: 59 - protein, 217 aa, artificial sequence
DIQMTQSPSSLSASVGDRVTITCRSSTGAVTTSNYANWVQQKPGKAPKGLIGGTNKRAPGVPSRFSGSLIGDKATLTISSLQPEDFATYYCALWYSNLWVFGQGTKVEIKRTVAAPSVFIFPPSDECLKSGTASVVCLLNNFYPREAKVQWKVDNALQSGNSQESVTEQDSKDSTYSLSSTLTLSKADYEKHKVYACEVTHQGLSSPVTKSFNRGES

SEQ ID NO: 60 - protein, 218 aa, artificial sequence
DIVMTQSPDSLAVSLGERATINCRASESVDSYGITFMNWYQKKPGQPPKLLIYAASNQGSGVPDRFSGSGSGTDFTLTISSLQAEDVAVYYCQQSKEVPWTFGQGTKLEIKRTVAAPSVFIFPPSDEQLKSGTASVVCLLNNFYPREAKVQWKVDNALQSGNSQESVTEQDSKDSTYSLSSTLTLSKADYEKHKVYACEVTHQGLSSPVTKSFNRGEC

SEQ ID NO: 61 - protein, 450 aa, artificial sequence
QVQLVQSGAEVKKPGASVKVSCKASGYTFIGYVMHWVRDAPGQGLEWMGYINPYNDVSQHQGKFKGRVTMTSDTSTSTVYMELSSLRSEDTAVYYCAREGRLGLRVLAYWGQGTLVTVSSASTKGPSVFPLAPSSKSTSGGTAALGCLVKDYFPEPVTVSWNSGALTSGVHTFPAVLQSSGLYSLSSVVTVPSSSLGTQTYICNVNHKPSNTKVDKKVEPKSCDKTHTCPPCPAPELLGGPSVFLFPPKPKDTLMISRTPEVTCVVVDVSHEDPEVKFNWYVDGVEVHNAKTKPREEQYNSTYRVVSVLTVLHQDWLNGKEYKCKVSNKALPAPIEKTISKAKGQPREPQVYTLPPSREEMTKNQVRLTCLVKGFYPSDIAVEWESNGQPENNYKTTPPVLKSDGSFFLYSKLTVDKSRWQQGNVFSCSVMHEALHNHYTQKSLSLSPGK

SEQ ID NO: 62 - protein, 688 aa, artificial sequence
QVQLVQSGAEVKKPGASVKVSCKASGYTFIGYVMHWVRDAPGQGLEWMGYINPYNDVSQHQGKFKGRVTMTSDTSTSTVYMELSSLRSEDTAVYYCAREGRLGLRVLAYWGQGTLVTVSSASTKGPSVFPLAPSSKSTSGGTAALGCLVKDYFPEPVTVSWNSGALTSGVHTFPAVLQSSGLYSLSSVVTVPSSSLGTQTYICNVNHKPSNTKVDKKVEPKSCGGGGSGGGGSEVQLVESGGGLVQPGGSLKLSCAASGFTFNTYAMNWVRKASGKGLEWVGRIRSKYNNYATYYADSVKDRFTISRDDSKSTLYLQMNSLKTEDTAVYYCARHGNFGQSYVSWFAYWGQGTTVTVSSASTKGPSVCPLAPSSKSTSGGTAALGCLVKDYFPEPVTVSWNSGALTSGVHTFPAVLQSSGLYSLSSVVTVPSSSLGTQTYICNVNHKPSNTKVDKKVEPKSSDKTHTCPPCPAPELLGGPSVFLFPPKPKDTLMISRTPEVTCVVVDVSHEDPEVKFNWYVDGVEVHNAKTKPREEQYNSTYRVVSVLTVLHQDWLNGKEYKCKVSNKALPAPIEKTISKAKGQPREPQVTTLPPSREEMTKNQVSLTCLVSGFYPSDIAVEWESNGQPENNYKTTPPVLDSDGSFFLYSDLTVDKSRWQQGNVFSCSVMHEALHNHYTQKSLSLSPGK

SEQ ID NO: 63 - protein, 217 aa, artificial sequence
DIQMTQSPSSLSASVGDRVTITCRSSTGAVTTSNYANWVQDKPGKAPKGLIGGTNKRAPGVPSRFSGSLIGDKATLTISSLQPEDFATYYCALWYSNLWVFGQGTKVEIKRTVAAPSVFIFPPSDECLKSGTASVVCLLNNFYPREAKVQWKVDNALQSGNSQESVTEQDSKDSTYSLSSTLTLSKADYEKHKVYACEVTHQGLSSPVTKSFNRGES

SEQ ID NO: 64 - protein, 688 aa, artificial sequence
QVQLVQSGAEVKKPGASVKVSCKASGYTFIGYVMHWVRQAPGQGLEWMGYINPYNDVSQHQGKFKGRVTMTSDTSTSTVYMELSSLRSEDTAVYYCAREGRLGLRVLAYWGQGTLVTVSSASTKGPSVFPLAPSSKSTSGGTAALGCLVKDYFPEPVTVSWNSGALTSGVHTFPAVLQSSGLYSLSSVVTVPSSSLGTQTYICNVNHKPSNTKVDKKVEPKSCDKTHTCPPCPAPELLGGPSVFLFPPKPKDTLMISRTPEVTCVVVDVSHEDPEVKFNWYVDGVEVHNAKTKPREEQYNSTYRVVSVLTVLHQDWLNGKEYKCKVSNKALPAPIEKTISKAKGQPREPQVTTLPPSREEMTKNQVSLTCLVSGFYPSDIAVEWESNGQPENNYKTTPPVLDSDGSFFLYSDLTVDKSRWQQGNVFSCSVMHEALHNHYTQKSLSLSPGKGGGGSGGGGSEVQLVESGGGLVQPGGSLKLSCAASGFTFNTYAMNWVRQASGKGLEWVGRIRSKYNNYATYYADSVKDRFTISRDDSKSTLYLQMNSLKTEDTAVYYCARHGNFGQSYVSWFAYWGQGTTVTVSSASTKGPSVCPLAPSSKSTSGGTAALGCLVKDYFPEPVTVSWNSGALTSGVHTFPAVLQSSGLYSLSSVVTVPSSSLGTQTYICNVNHKPSNTKVDKKVEPKSS

SEQ ID NO: 65 - protein, 688 aa, artificial sequence
QVQLVQSGAEVKKPGASVKVSCKASGYTFIGYVMHWVRDAPGQGLEWMGYINPYNDVSQHQGKFKGRVTMTSDTSTSTVYMELSSLRSEDTAVYYCAREGRLGLRVLAYWGQGTLVTVSSASTKGPSVFPLAPSSKSTSGGTAALGCLVKDYFPEPVTVSWNSGALTSGVHTFPAVLQSSGLYSLSSVVTVPSSSLGTQTYICNVNHKPSNTKVDKKVEPKSCDKTHTCPPCPAPELLGGPSVFLFPPKPKDTLMISRTPEVTCVVVDVSHEDPEVKFNWYVDGVEVHNAKTKPREEQYNSTYRVVSVLTVLHQDWLNGKEYKCKVSNKALPAPIEKTISKAKGQPREPQVTTLPPSREEMTKNQVSLTCLVSGFYPSDIAVEWESNGQPENNYKTTPPVLDSDGSFFLYSDLTVDKSRWQQGNVFSCSVMHEALHNHYTQKSLSLSPGKGGGGSGGGGSEVQLVESGGGLVQPGGSLKLSCAASGFTFNTYAMNWVRKASGKGLEWVGRIRSKYNNYATYYADSVKDRFTISRDDSKSTLYLQMNSLKTEDTAVYYCARHGNFGQSYVSWFAYWGQGTTVTVSSASTKGPSVCPLAPSSKSTSGGTAALGCLVKDYFPEPVTVSWNSGALTSGVHTFPAVLQSSGLYSLSSVVTVPSSSLGTQTYICNVNHKPSNTKVDKKVEPKSS

SEQ ID NO: 66 - protein, 688 aa, artificial sequence
QVQLVQSGAEVKKPGASVKVSCKASGYTFIGYVMHWVRQAPGQGLEWMGYINPYNDVSQHQGKFKGRVTMTSDTSTSTVYMELSSLRSEDTAVYYCAREGRLGLRVLAYWGQGTLVTVSSASTKGPSVFPLAPSSKSTSGGTAALGCLVKDYFPEPVTVSWNSGALTSGVHTFPAVLQSSGLYSLSSVVTVPSSSLGTQTYICNVNHKPSNTKVDKKVEPKSCDKTHTCPPCPAPELLGGPSVFLFPPKPKDTLMISRTPEVTCVVVDVSHEDPEVKFNWYVDGVEVHNAKTKPREEQYNSTYRVVSVLTVLHQDWLNGKEYKCKVSNKALPAPIEKTISKAKGQPREPQVYTLPPSREEMTKNQVSLTCLVKGFYPSDIAVEWESNGQPENNYKTTPPVLDSDGSFFLYSKLTVDKSRWQQGNVFSCSVMHEALHNHYTQKSLSLSPGKGGGGSGGGGSEVQLVESGGGLVQPGGSLKLSCAASGFTFNTYAMNWVRQASGKGLEWVGRIRSKYNNYATYYADSVKDRFTISRDDSKSTLYLQMNSLKTEDTAVYYCARHGNFGQSYVSWFAYWGQGTTVTVSSASTKGPSVCPLAPSSKSTSGGTAALGCLVKDYFPEPVTVSWNSGALTSGVHTFPAVLQSSGLYSLSSVVTVPSSSLGTQTYICNVNHKPSNTKVDKKVEPKSS

SEQ ID NO: 67 - protein, 688 aa, artificial sequence
QVQLVQSGAEVKKPGASVKVSCKASGYTFIGYVMHWVRDAPGQGLEWMGYINPYNDVSQHQGKFKGRVTMTSDTSTSTVYMELSSLRSEDTAVYYCAREGRLGLRVLAYWGQGTLVTVSSASTKGPSVFPLAPSSKSTSGGTAALGCLVKDYFPEPVTVSWNSGALTSGVHTFPAVLQSSGLYSLSSVVTVPSSSLGTQTYICNVNHKPSNTKVDKKVEPKSCDKTHTCPPCPAPELLGGPSVFLFPPKPKDTLMISRTPEVTCVVVDVSHEDPEVKFNWYVDGVEVHNAKTKPREEQYNSTYRVVSVLTVLHQDWLNGKEYKCKVSNKALPAPIEKTISKAKGQPREPQVYTLPPSREEMTKNQVSLTCLVKGFYPSDIAVEWESNGQPENNYKTTPPVLDSDGSFFLYSKLTVDKSRWQQGNVFSCSVMHEALHNHYTQKSLSLSPGKGGGGSGGGGSEVQLVESGGGLVQPGGSLKLSCAASGFTFNTYAMNWVRKASGKGLEWVGRIRSKYNNYATYYADSVKDRFTISRDDSKSTLYLQMNSLKTEDTAVYYCARHGNFGQSYVSWFAYWGQGTTVTVSSASTKGPSVCPLAPSSKSTSGGTAALGCLVKDYFPEPVTVSWNSGALTSGVHTFPAVLQSSGLYSLSSVVTVPSSSLGTQTYICNVNHKPSNTKVDKKVEPKSS

SEQ ID NO: 68 - protein, 450 aa, artificial sequence
QVQLVQSGAEVKKPGASVKVSCKASGYTFIGYVMHWVRQAPGQGLEWMGYINPYNDVSQHQGKFKGRVTMTSDTSTSTVYMELSSLRSEDTAVYYCAREGRLGLRVLAYWGQGTLVTVSSASTKGPSVFPLAPSSKSTSGGTAALGCLVKDYFPEPVTVSWNSGALTSGVHTFPAVLQSSGLYSLSSVVTVPSSSLGTQTYICNVNHKPSNTKVDKKVEPKSCDKTHTCPPCPAPEAAGGPSVFLFPPKPKDTLMISRTPEVTCVVVDVSHEDPEVKFNWYVDGVEVHNAKTKPREEQYNSTYRVVSVLTVLHQDWLNGKEYKCKVSNKALPAPIEKTISKAKGQPREPQVYTLPPSRDELTKNQVSLWCLVKGFYPSDIAVEWESNGQPENNYKTTPPVLDSDGSFFLYSKLTVDKSRWQQGNVFSCSVMHEALHNHYTQKSLSLSPGK

SEQ ID NO: 69 - protein, 705 aa, artificial sequence
EVQLVESGGGLVQPGGSLKLSCAASGFTFNTYAMNWVRQASGKGLEWVGRIRSKYNNYATYYADSVKDRFTISRDDSKSTLYLQMNSLKTEDTAVYYCARHYNFGQSYVSWFAYWGQGTTVTVSSASTKGPSVFPLAPSSKSTSGGTAALGCLVKDYFPEPVTVSWNSGALTSGVHTFPAVLQSSGLYSLSSVVTVPSSSLGTQTYICNVNHKPSNTKVDKKVEPKSCDKTHTCPPCPAPEAAGGPSVFLFPPKPKDTLMISRTPEVTCVVVDVSHEDPEVKFNWYVDGVEVHNAKTKPREEQYNSTYRVVSVLTVLHQDWLNGKEYKCKVSNKALPAPIEKTISKAKGQPREPQVYTLPPSRDELTKNQVSLSCAVKGFYPSDIAVEWESNGQPENNYKTTPPVLDSDGSFFLVSKLTVDKSRWQQGNVFSCSVMHEALHNHYTQKSLSLSPGAGGGGSGGGGSDIQMTQSPSSLSASVGDRVTITCRASQSISRYLNWYQQKPGKAPKLLIYAASSLQSGVPSRFSGSGSGTDFTLTISSLQPEDFATYYCQQKYFDITFGCGTKVEIKGGGGSGGGGSGGGGSQLQLQESGPGLVKPSETLSLTCTVSGGSIVSSSYYWTWIRQPPGKCLEWIGSISIAGSTYYNPSLKSRVTISVDTSKNQFSLKLSSVTAADTAVYYCARDRGDQILDVWSQGTMVTVSS

SEQ ID NO: 70 - protein, 215 aa, artificial sequence
QAVVTQEPSLTVSPGGTVTLTCRSSTGAVTTSNYANWVQQKPGQAPRGLIGGTNKRAPGVPARFSGSLLGDKAALTLLGAQPEDEAEYYCALWYSNLWVFGQGTKLTVLGQPKAAPSVTLFPPSSEELQANKATLVCLISDFYPGAVTVAWKADSSPVKAGVETTTPSKQSNNKYAASSYLSLTPEQWKSHRSYSCQVTHEGSTVEKTVAPTECS

SEQ ID NO: 71 - protein, 450 aa, artificial sequence
QVQLVQSGAEVKKPGASVKVSCKASGYTFIGYVMHWVRKAPGQGLEWMGYINPYNDVSQHQGKFKGRVTMTSDTSTSTVYMELSSLRSEDTAVYYCAREGRLGLRVLAYWGQGTLVTVSSASTKGPSVCPLAPSSKSTSGGTAALGCLVKDYFPEPVTVSWNSGALTSGVHTFPAVLQSSGLYSLSSVVTVPSSSLGTQTYICNVNHKPSNTKVDKKVEPKSSDKTHTCPPCPAPEAAGGPSVFLFPPKPKDTLMISRTPEVTCVVVDVSHEDPEVKFNWYVDGVEVHNAKTKPREEQYNSTYRVVSVLTVLHQDWLNGKEYKCKVSNKALPAPIEKTISKAKGQPREPQVYTLPPSRDELTKNQVSLWCLVKGFYPSDIAVEWESNGQPENNYKTTPPVLDSDGSFFLYSKLTVDKSRWQQGNVFSCSVMHEALHNHYTQKSLSLSPGK

SEQ ID NO: 72 - protein, 218 aa, artificial sequence
DIVMTQSPDSLAVSLGERATINCRASESVDSYGITFMNWYQDKPGQPPKLLIYAASNQGSGVPDRFSGSGSGTDFTLTISSLQAEDVAVYYCQQSKEVPWTFGQGTKLEIKRTVAAPSVFIFPPSDECLKSGTASVVCLLNNFYPREAKVQWKVDNALQSGNSQESVTEQDSKDSTYSLSSTLTLSKADYEKHKVYACEVTHQGLSSPVTKSFNRGES

SEQ ID NO: 73 - protein, 705 aa, artificial sequence
EVQLVESGGGLVQPGGSLKLSCAASGFTFNTYAMNWVRDASGKGLEWVGRIRSKYNNYATYYADSVKDRFTISRDDSKSTLYLQMNSLKTEDTAVYYCARHYNFGQSYVSWFAYWGQGTTVTVSSASTKGPSVFPLAPSSKSTSGGTAALGCLVKDYFPEPVTVSWNSGALTSGVHTFPAVLQSSGLYSLSSVVTVPSSSLGTQTYICNVNHKPSNTKVDKKVEPKSCDKTHTCPPCPAPEAAGGPSVFLFPPKPKDTLMISRTPEVTCVVVDVSHEDPEVKFNWYVDGVEVHNAKTKPREEQYNSTYRVVSVLTVLHQDWLNGKEYKCKVSNKALPAPIEKTISKAKGQPREPQVYTLPPSRDELTKNQVSLSCAVKGFYPSDIAVEWESNGQPENNYKTTPPVLDSDGSFFLVSKLTVDKSRWQQGNVFSCSVMHEALHNHYTQKSLSLSPGAGGGGSGGGGSDIQMTQSPSSLSASVGDRVTITCRASQSISRYLNWYQQKPGKAPKLLIYAASSLQSGVPSRFSGSGSGTDFTLTISSLQPEDFATYYCQQKYFDITFGCGTKVEIKGGGGSGGGGSGGGGSQLQLQESGPGLVKPSETLSLTCTVSGGSIVSSSYYWTWIRQPPGKCLEWIGSISIAGSTYYNPSLKSRVTISVDTSKNQFSLKLSSVTAADTAVYYCARDRGDQILDVWSQGTMVTVSS

SEQ ID NO: 74 - protein, 215 aa, artificial sequence
QAVVTQEPSLTVSPGGTVTLTCRSSTGAVTTSNYANWVQKKPGQAPRGLIGGTNKRAPGVPARFSGSLLGDKAALTLLGAQPEDEAEYYCALWYSNLWVFGQGTKLTVLGQPKAAPSVTLFPPSSEELQANKATLVCLISDFYPGAVTVAWKADSSPVKAGVETTTPSKQSNNKYAASSYLSLTPEQWKSHRSYSCQVTHEGSTVEKTVAPTECS

SEQ ID NO: 75 - protein, 120 aa, artificial sequence [sequence omitted]

SEQ ID NO: 76 - protein, 107 aa, artificial sequence [sequence omitted]

SEQ ID NO: 77 - protein, 119 aa, artificial sequence
EVRLLESGGGLVQPGGSLRLSCAASGFTFSNYAMGWVRQAPGKGLEWVSAISGSGGSTYYADSVKGRFTTSRDDSKNALYLQMNSLRAEDTAVYYCARGGPGWYAADVWGQGTTVTVSS

SEQ ID NO: 78 - protein, 107 aa, artificial sequence
DIQMTQSPSSLSASVGDRVTITCRASQSISSYLNWYQQKPGKAPKLLIYAASSLQSGVPSRFSGSGSGTDFTLTISSLQPEDFATYYCQQADLPAFAFGGGTKVEIK

SEQ ID NO: 79 - protein, 120 aa, artificial sequence
QVQLVQSGAEVKKPGSSVKVSCKASGGTFSSYAISWVRQAPGQGLEWMGLIIPMFDTAGYAQKFQGRVAITVDESTSTAYMELSSLRSEDTAVYYCARAEHSSTGTFDYWGQGTLVTVSS

SEQ ID NO: 80 - protein, 107 aa, artificial sequence
DIQMTQSPSSVSASVGDRVTITCRASQGISSWLAWYQQKPGKAPKLLISAASSLQSGVPSRFSGSGSGTDFTLTISSLQPEDFATYYCQQANHLPFTFGGGTKVEIK

SEQ ID NO: 81 - protein, 115 aa, artificial sequence
QVQLQESGPGLVKPSETLSLTCTVSGGSISSYYWSWIRQPPGKGLEWIGYIYYSGSTNYNPSLKSRVTISVDTSKNQFSLKLSSVTAADTAVYYCARGKTGSAAWGQGTLVTVSS

SEQ ID NO: 82 - protein, 107 aa, artificial sequence
DIQMTQSPSSVSASVGDRVTITCRASQGISRWLAWYQQKPGKAPKLLIYAASSLQSGVPSRFSGSGSGTDFTLTISSLQPEDFATYYCQQTVSFPITFGGGTKVEIK

SEQ ID NO: 83 - protein, 111 aa, artificial sequence
DIVMTQSPDSLAVSLGERATINCRASESVDSYGITFMNWYQQKPGQPPKLLIYAASNQGSGVPDRFSGSGSGTDFTLTISSLQAEDVAVYYCQQSKEVPWTFGQGTKLEIK

SEQ ID NO: 84 - protein, 15 aa, artificial sequence
RASESVDSYGITFMN

SEQ ID NO: 85 - protein, 7 aa, artificial sequence
AASNQGS

SEQ ID NO: 86 - protein, 9 aa, artificial sequence
QQSKEVPWT

SEQ ID NO: 87 - protein, 120 aa, artificial sequence
QVQLVQSGAEVKKPGASVKVSCKASGYTFIGYVMHWVRQAPGQGLEWMGYINPYNDVSQHQGKFKGRVTMTSDTSTSTVYMELSSLRSEDTAVYYCAREGRLGLRVLAYWGQGTLVTVSS

SEQ ID NO: 88 - protein, 5 aa, artificial sequence
GYVMH

SEQ ID NO: 89 - protein, 17 aa, artificial sequence
YINPYNDVSQHQGKFKG

SEQ ID NO: 90 - protein, 11 aa, artificial sequence
EGRLGLRVLAY

SEQ ID NO: 91 - protein, 125 aa, artificial sequence
EVQLVESGGGLVQPGGSLKLSCAASGFTFNTYAMNWVRQASGKGLEWVGRIRSKYNNYATYYADSVKDRFTISRDDSKSTLYLQMNSLKTEDTAVYYCARHGNFGQSYVSWFAYWGQGTTVTVSS

SEQ ID NO: 92 - protein, 110 aa, artificial sequence
DIQMTQSPSSLSASVGDRVTITCRSSTGAVTTSNYANWVQQKPGKAPKGLIGGTNKRAPGVPSRFSGSLIGDKATLTISSLQPEDFATYYCALWYSNLWVFGQGTKVEIK

SEQ ID NO: 93 - protein, 111 aa, artificial sequence
DIVMTQSPDSLAVSLGERATINCRASESVDSYGITFMNWYQKKPGQPPKLLIYAASNQGSGVPDRFSGSGSGTDFTLTISSLQAEDVAVYYCQQSKEVPWTFGQGTKLEIK

SEQ ID NO: 94 - protein, 120 aa, artificial sequence
QVQLVQSGAEVKKPGASVKVSCKASGYTFIGYVMHWVRDAPGQGLEWMGYINPYNDVSQHQGKFKGRVTMTSDTSTSTVYMELSSLRSEDTAVYYCAREGRLGLRVLAYWGQGTLVTVSS

SEQ ID NO: 95 - protein, 120 aa, artificial sequence; identical to SEQ ID NO: 94

SEQ ID NO: 96 - protein, 125 aa, artificial sequence
EVQLVESGGGLVQPGGSLKLSCAASGFTFNTYAMNWVRKASGKGLEWVGRIRSKYNNYATYYADSVKDRFTISRDDSKSTLYLQMNSLKTEDTAVYYCARHGNFGQSYVSWFAYWGQGTTVTVSS

SEQ ID NO: 97 - protein, 110 aa, artificial sequence
DIQMTQSPSSLSASVGDRVTITCRSSTGAVTTSNYANWVQDKPGKAPKGLIGGTNKRAPGVPSRFSGSLIGDKATLTISSLQPEDFATYYCALWYSNLWVFGQGTKVEIK

SEQ ID NO: 98 - protein, 107 aa, artificial sequence
RTVAAPSVCIFPPSDEQLKSGTASVVCLLNNFYPREAKVQWKVDNALQSGNSQESVTEQDSKDSTYSLSSTLTLSKADYEKHKVYACEVTHQGLSSPVTKSFNRGES

SEQ ID NO: 99 - protein, 107 aa, artificial sequence
RTVAAPCVFIFPPSDEQLKSGTASVVCLLNNFYPREAKVQWKVDNALQSGNSQESVTEQDSKDSTYSLSSTLTLSKADYEKHKVYACEVTHQGLSSPVTKSFNRGEC

SEQ ID NO: 100 - protein, 107 aa, artificial sequence
RTVAAPCVFIFPPSDEQLKSGTASVVCLLNNFYPREAKVQWKVDNALQSGNSQESVTEQDSKDSTYSLSSTLTLSKADYEKHKVYACEVTHQGLSSPVTKSFNRGES

SEQ ID NO: 101 - protein, 227 aa, artificial sequence
DKTHTCPPCPAPELLGGPSVFLFPPKPKDTLMISRTPEVTCVVVDVSHEDPEVKFNWYVDGVEVHNAKTKPREEQYNSTYRVVSVLTVLHQDWLNGKEYKCKVSNKALPAPIEKTISKAKGQPREPQVYTLPPSRDELTKNQVSLSCAVKGFYPSDIAVEWESNGQPENNYKTTPPVLDSDGSFFLVSKLTVDKSRWQQGNVFSCSVMHEALHNHYTQKSLSLSPGK

SEQ ID NO: 102 - protein, 125 aa, artificial sequence
EVQLVESGGGLVQPGGSLKLSCAASGFTFNTYAMNWVRQASGKGLEWVGRIRSKYNNYATYYADSVKDRFTISRDDSKSTLYLQMNSLKTEDTAVYYCARHYNFGQSYVSWFAYWGQGTTVTVSS

SEQ ID NO: 103 - protein, 119 aa, artificial sequence
QLQLQESGPGLVKPSETLSLTCTVSGGSIVSSSYYWTWIRQPPGKCLEWIGSISIAGSTYYNPSLKSRVTISVDTSKNQFSLKLSSVTAADTAVYYCARDRGDQILDVWSQGTMVTVSS

SEQ ID NO: 104 - protein, 7 aa, artificial sequence
SSSYYWT

SEQ ID NO: 105 - protein, 16 aa, artificial sequence
SISIAGSTYYNPSLKS

SEQ ID NO: 106 - protein, 9 aa, artificial sequence
DRGDQILDV

SEQ ID NO: 107 - protein, 106 aa, artificial sequence
DIQMTQSPSSLSASVGDRVTITCRASQSISRYLNWYQQKPGKAPKLLIYAASSLQSGVPSRFSGSGSGTDFTLTISSLQPEDFATYYCQQKYFDITFGCGTKVEIK

SEQ ID NO: 108 - protein, 11 aa, artificial sequence
RASQSISRYLN

SEQ ID NO: 109 - protein, 7 aa, artificial sequence
AASSLQS

SEQ ID NO: 110 - protein, 8 aa, artificial sequence
QQKYFDIT

SEQ ID NO: 111 - protein, 240 aa, artificial sequence
DIQMTQSPSSLSASVGDRVTITCRASQSISRYLNWYQQKPGKAPKLLIYAASSLQSGVPSRFSGSGSGTDFTLTISSLQPEDFATYYCQQKYFDITFGCGTKVEIKGGGGSGGGGSGGGGSQLQLQESGPGLVKPSETLSLTCTVSGGSIVSSSYYWTWIRQPPGKCLEWIGSISIAGSTYYNPSLKSRVTISVDTSKNQFSLKLSSVTAADTAVYYCARDRGDQILDVWSQGTMVTVSS

SEQ ID NO: 112 - protein, 109 aa, artificial sequence
QAVVTQEPSLTVSPGGTVTLTCRSSTGAVTTSNYANWVQQKPGQAPRGLIGGTNKRAPGVPARFSGSLLGDKAALTLLGAQPEDEAEYYCALWYSNLWVFGQGTKLTVL

SEQ ID NO: 113 - protein, 120 aa, artificial sequence
QVQLVQSGAEVKKPGASVKVSCKASGYTFIGYVMHWVRKAPGQGLEWMGYINPYNDVSQHQGKFKGRVTMTSDTSTSTVYMELSSLRSEDTAVYYCAREGRLGLRVLAYWGQGTLVTVSS

SEQ ID NO: 114 - protein, 125 aa, artificial sequence
EVQLVESGGGLVQPGGSLKLSCAASGFTFNTYAMNWVRDASGKGLEWVGRIRSKYNNYATYYADSVKDRFTISRDDSKSTLYLQMNSLKTEDTAVYYCARHYNFGQSYVSWFAYWGQGTTVTVSS

SEQ ID NO: 115 - protein, 109 aa, artificial sequence
QAVVTQEPSLTVSPGGTVTLTCRSSTGAVTTSNYANWVQKKPGQAPRGLIGGTNKRAPGVPARFSGSLLGDKAALTLLGAQPEDEAEYYCALWYSNLWVFGQGTKLTVL

SEQ ID NO: 116 - protein, 103 aa, artificial sequence
ASTKGPSVFPLAPSSKSTSGGTAALGCLVKDYFPEPVTVSWNSGALTSGVHTFPAVLQSSGLYSLSSVVTVPSSSLGTQTYICNVNHKPSNTKVDKKVEPKSC

SEQ ID NO: 117 - protein, 110 aa, artificial sequence
APELLGGPSVFLFPPKPKDTLMISRTPEVTCVVVDVSHEDPEVKFNWYVDGVEVHNAKTKPREEQYNSTYRVVSVLTVLHQDWLNGKEYKCKVSNKALPAPIEKTISKAK

SEQ ID NO: 118 - protein, 107 aa, artificial sequence
GQPREPQVYTLPPSRDELTKNQVSLTCLVKGFYPSDIAVEWESNGQPENNYKTTPPVLDSDGSFFLYSKLTVDKSRWQQGNVFSCSVMHEALHNHYTQKSLSLSPGK

SEQ ID NO: 119 - protein, 10 aa, artificial sequence
  SITE 8: note = X may be X or P
DKTHTCPXCP

SEQ ID NO: 120 - protein, 7 aa, artificial sequence
  SITE 5: note = X may be S or P
HTCPXCP

SEQ ID NO: 121 - protein, 5 aa, artificial sequence
  SITE 3: note = X may be S or P
CPXCP

SEQ ID NO: 122 - protein, 227 aa, artificial sequence
DKTHTCPPCPAPELLGGPSVFLFPPKPKDTLMISRTPEVTCVVVDVSHEDPEVKFNWYVDGVEVHNAKTKPREEQYNSTYRVVSVLTVLHQDWLNGKEYKCKVSNKALPAPIEKTISKAKGQPREPQVYTLPPSRDELTKNQVSLTCLVKGFYPSDIAVEWESNGQPENNYKTTPPVLDSDGSFFLYSKLTVDKSRWQQGNVFSCSVMHEALHNHYTQKSLSLSPGK

SEQ ID NO: 123 - protein, 225 aa, artificial sequence
PPCPSCPAPEFLGGPSVFLFPPKPKDTLMISRTPEVTCVVVDVSQEDPEVQFNWYVDGVEVHNAKTKPREEQFNSTYRVVSVLTVLHQDWLNGKEYKCKVSNKGLPSSIEKTISKAKGQPREPQVYTLPPSQEEMTKNQVSLTCLVKGFYPSDIAVEWESNGQPENNYKTTPPVLDSDGSFFLYSRLTVDKSRWQEGNVFSCSVMHEAVLHNHYTQKSLSLSLGK

SEQ ID NO: 124 - protein, 227 aa, artificial sequence
DKTHTCPPCPAPEAAGGPSVFLFPPKPKDTLMISRTPEVTCVVVDVSHEDPEVKFNWYVDGVEVHNAKTKPREEQYNSTYRVVSVLTVLHQDWLNGKEYKCKVSNKALPAPIEKTISKAKGQPREPQVCTLPPSRDELTKNQVSLSCAVKGFYPSDIAVEWESNGQPENNYKTTPPVLDSDGSFFLVSKLTVDKSRWQQGNVFSCSVMHEALHNHYTQKSLSLSPGK

SEQ ID NO: 125 - protein, 227 aa, artificial sequence
DKTHTCPPCPAPEAAGGPSVFLFPPKPKDTLMISRTPEVTCVVVDVSHEDPEVKFNWYVDGVEVHNAKTKPREEQYNSTYRVVSVLTVLHQDWLNGKEYKCKVSNKALPAPIEKTISKAKGQPREPQVYTLPPCRDELTKNQVSLWCLVKGFYPSDIAVEWESNGQPENNYKTTPPVLDSDGSFFLYSKLTVDKSRWQQGNVFSCSVMHEALHNHYTQKSLSLSPGK

SEQ ID NO: 126 - protein, 227 aa, artificial sequence
DKTHTCPPCPAPELLGGPSVFLFPPKPKDTLMISRTPEVTCVVVDVSHEDPEVKFNWYVDGVEVHNAKTKPREEQYNSTYRVVSVLTVLHQDWLNGKEYKCKVSNKALPAPIEKTISKAKGQPREPQVYTLPPSREEMTKNQVRLTCLVKGFYPSDIAVEWESNGQPENNYKTTPPVLKSDGSFFLYSKLTVDKSRWQQGNVFSCSVMHEALHNHYTQKSLSLSPGK

SEQ ID NO: 127 - protein, 227 aa, artificial sequence
DKTHTCPPCPAPELLGGPSVFLFPPKPKDTLMISRTPEVTCVVVDVSHEDPEVKFNWYVDGVEVHNAKTKPREEQYNSTYRVVSVLTVLHQDWLNGKEYKCKVSNKALPAPIEKTISKAKGQPREPQVTTLPPSREEMTKNQVSLTCLVSGFYPSDIAVEWESNGQPENNYKTTPPVLDSDGSFFLYSDLTVDKSRWQQGNVFSCSVMHEALHNHYTQKSLSLSPGK

SEQ ID NO: 128 - protein, 107 aa, artificial sequence
RTVAAPSVFIFPPSDECLKSGTASVVCLLNNFYPREAKVQWKVDNALQSGNSQESVTEQDSKDSTYSLSSTLTLSKADYEKHKVYACEVTHQGLSSPVTKSFNRGES

SEQ ID NO: 129 - protein, 103 aa, artificial sequence
ASTKGPSVCPLAPSSKSTSGGTAALGCLVKDYFPEPVTVSWNSGALTSGVHTFPAVLQSSGLYSLSSVVTVPSSSLGTQTYICNVNHKPSNTKVDKKVEPKSS

SEQ ID NO: 130 - protein, 227 aa, artificial sequence
DKTHTCPPCPAPEAAGGPSVFLFPPKPKDTLMISRTPEVTCVVVDVSHEDPEVKFNWYVDGVEVHNAKTKPREEQYNSTYRVVSVLTVLHQDWLNGKEYKCKVSNKALPAPIEKTISKAKGQPREPQVYTLPPSRDELTKNQVSLSCAVKGFYPSDIAVEWESNGQPENNYKTTPPVLDSDGSFFLVSKLTVDKSRWQQGNVFSCSVMHEALHNHYTQKSLSLSPGK

SEQ ID NO: 131 - protein, 227 aa, artificial sequence
DKTHTCPPCPAPEAAGGPSVFLFPPKPKDTLMISRTPEVTCVVVDVSHEDPEVKFNWYVDGVEVHNAKTKPREEQYNSTYRVVSVLTVLHQDWLNGKEYKCKVSNKALPAPIEKTISKAKGQPREPQVYTLPPSRDELTKNQVSLWCLVKGFYPSDIAVEWESNGQPENNYKTTPPVLDSDGSFFLYSKLTVDKSRWQQGNVFSCSVMHEALHNHYTQKSLSLSPGK

SEQ ID NO: 132 - protein, 103 aa, artificial sequence
ASTKGPSVFPLAPSSKSTSGGTAALGCLVKDYFPEPVTVSWNSGALTSGVCTFPAVLQSSGLYSLSSVVTVPSSSLGTQTYICNVNHKPSNTKVDKKVEPKSC

SEQ ID NO: 133 - protein, 103 aa, artificial sequence
ASTKGPSVFPLAPSSKSTSGGTAALGCLVKDYFPEPVTVSWNSGALTSGVCTFPAVLQSSGLYSLSSVVTVPSSSLGTQTYICNVNHKPSNTKVDKKVEPKSS

SEQ ID NO: 134 - protein, 103 aa, artificial sequence
ASTKGPSVFPLAPSSKSTSGGTAALGCLVKDYFPEPVTVSWNSGALTSGVHTCPAVLQSSGLYSLSSVVTVPSSSLGTQTYICNVNHKPSNTKVDKKVEPKSC

SEQ ID NO: 135 - protein, 103 aa, artificial sequence
ASTKGPSVFPLAPSSKSTSGGTAALGCLVKDYFPEPVTVSWNSGALTSGVHTCPAVLQSSGLYSLSSVVTVPSSSLGTQTYICNVNHKPSNTKVDKKVEPKSS

SEQ ID NO: 136 - protein, 103 aa, artificial sequence
ASTKGPSVFPLAPSSKSTSGGTAALGCLVKDYFPEPVTVSWNSGALTSGVHTFPACLQSSGLYSLSSVVTVPSSSLGTQTYICNVNHKPSNTKVDKKVEPKSC

SEQ ID NO: 137 - protein, 103 aa, artificial sequence
ASTKGPSVFPLAPSSKSTSGGTAALGCLVKDYFPEPVTVSWNSGALTSGVHTFPACLQSSGLYSLSSVVTVPSSSLGTQTYICNVNHKPSNTKVDKKVEPKSS

SEQ ID NO: 138 - protein, 103 aa, artificial sequence
ASTKGPSVFPCAPSSKSTSGGTAALGCLVKDYFPEPVTVSWNSGALTSGVHTFPAVLQSSGLYSLSSVVTVPSSSLGTQTYICNVNHKPSNTKVDKKVEPKSC

SEQ ID NO: 139 - protein, 103 aa, artificial sequence
ASTKGPSVFPCAPSSKSTSGGTAALGCLVKDYFPEPVTVSWNSGALTSGVHTFPAVLQSSGLYSLSSVVTVPSSSLGTQTYICNVNHKPSNTKVDKKVEPKSS

SEQ ID NO: 140 - protein, 103 aa, artificial sequence
ASTKGPSVFPLAPSSKCTSGGTAALGCLVKDYFPEPVTVSWNSGALTSGVHTFPAVLQSSGLYSLSSVVTVPSSSLGTQTYICNVNHKPSNTKVDKKVEPKSC

SEQ ID NO: 141 - protein, 103 aa, artificial sequence
ASTKGPSVFPLAPSSKCTSGGTAALGCLVKDYFPEPVTVSWNSGALTSGVHTFPAVLQSSGLYSLSSVVTVPSSSLGTQTYICNVNHKPSNTKVDKKVEPKSS

SEQ ID NO: 142 - protein, 103 aa, artificial sequence
ASTKGPSVFPLAPSSKSTCGGTAALGCLVKDYFPEPVTVSWNSGALTSGVHTFPAVLQSSGLYSLSSVVTVPSSSLGTQTYICNVNHKPSNTKVDKKVEPKSC

SEQ ID NO: 143 - protein, 103 aa, artificial sequence
ASTKGPSVFPLAPSSKSTCGGTAALGCLVKDYFPEPVTVSWNSGALTSGVHTFPAVLQSSGLYSLSSVVTVPSSSLGTQTYICNVNHKPSNTKVDKKVEPKSS

SEQ ID NO: 144 - protein, 103 aa, artificial sequence
ASTKGPSVFPLAPSSKSTSGGTAALGCLVKDYFPEPVTVSWNSGALTSGVHTFCAVLQSSGLYSLSSVVTVPSSSLGTQTYICNVNHKPSNTKVDKKVEPKSC

SEQ ID NO: 145 - protein, 103 aa, artificial sequence
ASTKGPSVFPLAPSSKSTSGGTAALGCLVKDYFPEPVTVSWNSGALTSGVHTFCAVLQSSGLYSLSSVVTVPSSSLGTQTYICNVNHKPSNTKVDKKVEPKSS

SEQ ID NO: 146 - protein, 103 aa, artificial sequence
ASTKGPSVFPLAPSSKSTSGGCAALGCLVKDYFPEPVTVSWNSGALTSGVHTFPAVLQSSGLYSLSSVVTVPSSSLGTQTYICNVNHKPSNTKVDKKVEPKSC

SEQ ID NO: 147 - protein, 103 aa, artificial sequence
ASTKGPSVFPLAPSSKSTSGGCAALGCLVKDYFPEPVTVSWNSGALTSGVHTFPAVLQSSGLYSLSSVVTVPSSSLGTQTYICNVNHKPSNTKVDKKVEPKSS

SEQ ID NO: 148 - protein, 107 aa, artificial sequence
RTVAAPSVFIFPPSDEQLKSGTASVVCLLNNFYPREAKVQWKVDNALQSGNSQESVCEQDSKDSTYSLSSTLTLSKADYEKHKVYACEVTHQGLSSPVTKSFNRGEC

SEQ ID NO: 149 - protein, 107 aa, artificial sequence
RTVAAPSVFIFPPSDEQLKSGTASVVCLLNNFYPREAKVQWKVDNALQSGNSQESVCEQDSKDSTYSLSSTLTLSKADYEKHKVYACEVTHQGLSSPVTKSFNRGES

SEQ ID NO: 150 - protein, 107 aa, artificial sequence
RTVAAPSVFIFPPSDEQLKSGTASVVCLLNNFYPREAKVQWKVDNALQSGNSQECVTEQDSKDSTYSLSSTLTLSKADYEKHKVYACEVTHQGLSSPVTKSFNRGEC

SEQ ID NO: 151 - protein, 107 aa, artificial sequence
RTVAAPSVFIFPPSDEQLKSGTASVVCLLNNFYPREAKVQWKVDNALQSGNSQECVTEQDSKDSTYSLSSTLTLSKADYEKHKVYACEVTHQGLSSPVTKSFNRGES

SEQ ID NO: 152 - protein, 107 aa, artificial sequence
RTVAAPSVFIFPPSDEQLKSGTASVVCLLNNFYPREAKVQWKVDNALQSGNSCESVTEQDSKDSTYSLSSTLTLSKADYEKHKVYACEVTHQGLSSPVTKSFNRGEC